European Patent Application EP 4 324 843 A1, published February 21, 2024. Title: Production of CRM197. Applicant: SenseUp GmbH. The sequence listing filed with the application follows.

SEQUENCE LISTING (8 sequences)

SEQ ID NO: 1 - DNA, 105 bp, Bacillus subtilis
  source 1..105: mol_type = other DNA
atgaaaatcagtatgcaaaaagcagatttttggaaaaaagcagcgatctcattacttgttttcaccatgttttttaccctgatgatgagcgaaacggtttttgcg

SEQ ID NO: 2 - protein, 535 aa, synthetic construct
GADDVVDSSKSFVMENFSSYHGTKPGYVDSIQKGIQKPKSGTQGNYDDDWKEFYSTDNKYDAAGYSVDNENPLSGKAGGVVKVTYPGLTKVLALKVDNAETIKKELGLSLTEPLMEQVGTEEFIKRFGDGASRVVLSLPFAEGSSSVEYINNWEQAKALSVELEINFETRGKRGQDAMYEYMAQACAGNRVRRSVGSSLSCINLDWDVIRDKTKTKIESLKEHGPIKNKMSESPNKTVSEEKAKQYLEEFHQTALEHPELSELKTVTGTNPVFAGANYAAWAVNVAQVIDSETADNLEKTTAALSILPGIGSVMGIADGAVHHNTEEIVAQSIALSSLMVAQAIPLVGELVDIGFAAYNFVESIINLFQVVHNSYNRPAYSPGHKTQPFLHDGYAVSWNTVEDSIIRTGFQGESGHDIKITAENTPLPIAGVLLPTIPGKLDVNKSKTHISVNGRKIRMRCRAIDGDVTFCRPKSPVYVGNGVHANLHVAFHRSSSEKIHSNEISSDSIGVLGYQKTVDHTKVNSKLSLFFEIKS

SEQ ID NO: 3 - DNA, 1605 bp, synthetic construct
  source 1..1605: mol_type = other DNA
ggcgctgacgacgttgttgactcctccaagtccttcgttatggagaacttctcctcctaccacggcaccaagccaggctacgttgactccatccagaagggcatccagaagccaaagtccggcacccagggcaactacgacgacgactggaaggagttctactccaccgacaacaagtacgacgctgctggctactccgttgacaacgagaacccactgtccggcaaggctggcggcgttgttaaggttacctacccaggcctgaccaaggttctggctctgaaggttgacaacgctgagaccatcaagaaggagctgggcctgtccctgaccgagccactgatggagcaggttggcaccgaggagttcatcaagcgcttcggcgacggcgcttcccgcgttgttctgtccctgccattcgctgagggctcctcctccgttgagtacatcaacaactgggagcaggctaaggctctgtccgttgagctggagatcaacttcgagacccgcggcaagcgcggccaggacgctatgtacgagtacatggctcaggcttgcgctggcaaccgcgttcgccgctccgttggctcctccctgtcctgcatcaacctggactgggacgttatccgcgacaagaccaagaccaagatcgagtccctgaaggagcacggcccaatcaagaacaagatgtccgagtccccaaacaagaccgtttccgaggagaaggctaagcagtacctggaggagttccaccagaccgctctggagcacccagagctgtccgagctgaagaccgttaccggcaccaacccagttttcgctggcgctaactacgctgcttgggctgttaacgttgctcaggttatcgactccgagaccgctgacaacctggagaagaccaccgctgctctgtccatcctgccaggcatcggctccgttatgggcatcgctgacggcgctgttcaccacaacaccgaggagatcgttgctcagtccatcgctctgtcctccctgatggttgctcaggctatcccactggttggcgagctggttgacatcggcttcgctgcttacaacttcgttgagtccatcatcaacctgttccaggttgttcacaactcctacaaccgcccagcttactccccaggccacaagacccagccattcctgcacgacgggtacgctgtcagctggaacaccgttgaggactccatcatccgcaccggcttccagggcgagtccggccacgacatcaagatcaccgctgagaacaccccactgccaatcgctggcgttctgctgccaaccatcccaggcaagctggacgttaacaagtccaagacccacatctccgttaacggccgcaagatccgcatgcgctgccgcgctatcgacggcgacgttaccttctgccgcccaaagtccccagtttacgttggcaacggcgttcacgctaacctgcacgttgctttccaccgctcctcctccgagaagatccactccaacgagatctcctccgactccatcggcgttctgggctaccagaagaccgttgaccacaccaaggttaactccaagctgtccctgttcttcgagatcaagtcc

SEQ ID NO: 4 - DNA, 9642 bp, synthetic construct
  source 1..9642: mol_type = other DNA
atgaaaatcagtatgcaaaaagcagatttttggaaaaaagcagcgatctcattacttgttttcaccatgttttttaccctgatgatgagcgaaacggtttttgcgggcgctgacgacgttgttgactcctccaagtccttcgttatggagaacttctcctcctaccacggcaccaagccaggctacgttgactccatccagaagggcatccagaagccaaagtccggcacccagggcaactacgacgacgactggaaggagttctactccaccgacaacaagtacgacgctgctggctactccgttgacaacgagaacccactgtccggcaaggctggcggcgttgttaaggttacctacccaggcctgaccaaggttctggctctgaaggttgacaacgctgagaccatcaagaaggagctgggcctgtccctgaccgagccactgatggagcaggttggcaccgaggagttcatcaagcgcttcggcgacggcgcttcccgcgttgttctgtccctgccattcgctgagggctcctcctccgttgagtacatcaacaactgggagcaggctaaggctctgtccgttgagctggagatcaacttcgagacccgcggcaagcgcggccaggacgctatgtacgagtacatggctcaggcttgcgctggcaaccgcgttcgccgctccgttggctcctccctgtcctgcatcaacctggactgggacgttatccgcgacaagaccaagaccaagatcgagtccctgaaggagcacggcccaatcaagaacaagatgtccgagtccccaaacaagaccgtttccgaggagaaggctaagcagtacctggaggagttccaccagaccgctctggagcacccagagctgtccgagctgaagaccgttaccggcaccaacccagttttcgctggcgctaactacgctgcttgggctgttaacgttgctcaggttatcgactccgagaccgctgacaacctggagaagaccaccgctgctctgtccatcctgccaggcatcggctccgttatgggcatcgctgacggcgctgttcaccacaacaccgaggagatcgttgctcagtccatcgctctgtcctccctgatggttgctcaggctatcccactggttggcgagctggttgacatcggcttcgctgcttacaacttcgttgagtccatcatcaacctgttccaggttgttcacaactcctacaaccgcccagcttactccccaggccacaagacccagccattcctgcacgacgggtacgctgtcagctggaacaccgttgaggactccatcatccgcaccggcttccagggcgagtccggccacgacatcaagatcaccgctgagaacaccccactgccaatcgctggcgttctgctgccaaccatcccaggcaagctggacgttaacaagtccaagacccacatctccgttaacggccgcaagatccgcatgcgctgccgcgctatcgacggcgacgttaccttctgccgcccaaagtccccagtttacgttggcaacggcgttcacgctaacctgcacgttgctttccaccgctcctcctccgagaagatccactccaacgagatctcctccgactccatcggcgttctgggctaccagaagaccgttgaccacaccaaggttaactccaagctgtccctgttcttcgagatcaagtcctaaggatccccgggtaccgagctcgaatacactggccgtcgttttacagccaagcttggctgttttggcggatgagagaagattttcagcctgatacagattaaatcagaacgcagaagcggtctgataaaacagaatttgcctggcggcagtagcgcggtggtcccacctgaccccatgccgaactcagaagtgaaacgccgtagcgccgatggtagtgtggggtctccccatgcgagagtagggaactgccaggcatcaaataaaacgaaaggctcagtcgaaagactgggcctttcgttttatctgttgtttgtcggtgaacgctctcctgagtaggacaaatccgccgggagcggatttgaacgttgcgaagcaacggcccggagggtggcgggcaggacgcccgccataaactgccaggcatcaaattaagcagaaggccatcctgacggatggcctttttgcgtttctacaaactcttttgtttatttttctaaatacattcaaatatgtatccgctcatgagacaataaccctgataaatgcttcaataatattgaaaaaggaagagtatgagtattcaacatttccgtgtcgcccttattcccttttttgcggcattttgccttcctgtttttgctcacccagaaacgctggtgaaagtaaaagatgctgaagatcagttgggtgcacgagtgggttacatcgaactggatctcaacagcggtaagatccttgagagttttcgccccgaagaacgttttccaatgatgagcacttttaaagttctgctatgtggcgcggtattatcccgtgttgacgccgggcaagagcaactcggtcgccgcatacactattctcagaatgacttggttgagtaattcgtaatcatgtcataggctcttccgcttcctcgctcactgactcgctgcgctcggtcgttcggctgcggcgagcggtatcagctcactcaaaggcggtaatacggttatccacagaatcaggggataacgcaggaaagaacatgtgagcaaaaggccagcaaaaggccaggaaccgtaaaaaggccgcgttgctggcgtttttccataggctccgcccccctgacgagcatcacaaaaatcgacgctcaagtcagaggtggcgaaacccgacaggactataaagataccaggcgtttccccctggaagctccctcgtgcgctctcctgttccgaccctgccgcttaccggatacctgtccgcctttctcccttcgggaagcgtggcgctttctcatagctcacgctgtaggtatctcagttcggtgtaggtcgttcgctccaagctgggctgtgtgcacgaaccccccgttcagcccgaccgctgcgccttatccggtaactatcgtcttgagtccaacccggtaagacacgacttatcgccactggcagcagccactggtaacaggattagcagagcgaggtatgtaggcggtgctacagagttcttgaagtggtggcctaactacggctacactagaagaacagtatttggtatctgcgctctgctgaagccagttaccttcggaaaaagagttggtagctcttgatccggcaaacaaaccaccgctggtagcggtggtttttttgtttgcaagcagcagattacgcgcagaaaaaaaggatctcaagaagatcctttgatcttttctacggggtctgacgctcagtggaacgaaaactcacgttaagggattttggtcatgagattatcaaaaaggatcttcacctagatccttttggggggggggggaaagccacgttgtgtctcaaaatctctgatgttacattgcacaagataaaaatatatcatcatgaacaataaaactgtctgcttacataaacagtaatacaaggggtgttatgagccatattcaacgggaaacgtcttgctcgaggccgcgattaaattccaacatggatgctgatttatatgggtataaatgggctcgcgataatgtcgggcaatcaggtgcgacaatctatcgattgtatgggaagcccgatgcgccagagttgtttctgaaacatggcaaaggtagcgttgccaatgatgttacagatgagatggtcagactaaactggctgacggaatttatgcctcttccgaccatcaagcattttatccgtactcctgatgatgcatggttactcaccactgcgatccccgggaaaacagcattccaggtattagaagaatatcctgattcaggtgaaaatattgttgatgcgctggcagtgttcctgcgccggttgcattcgattcctgtttgtaattgtccttttaacagcgatcgcgtatttcgtctcgctcaggcgcaatcacgaatgaataacggtttggttgatgcgagtgattttgatgacgagcgtaatggctggcctgttgaacaagtctggaaagaaatgcataagcttttgccattctcaccggattcagtcgtcactcatggtgatttctcacttgataaccttatttttgacgaggggaaattaataggttgtattgatgttggacgagtcggaatcgcagaccgataccaggatcttgccatcctatggaactgcctcggtgagttttctccttcattacagaaacggctttttcaaaaatatggtattgataatcctgatatgaataaattgcagtttcatttgatgctcgatgagtttttctaatcagaattggttaattggttgtaacactggcagagcattacgctgacttgacgggacggcggctttgttgaataaatcgaacttttgctgagttgaaggatcagatcacgcatcttcccgacaacgcagaccgttccgtggcaaagcaaaagttcaaaatcaccaactggtccacctacaacaaagctctcatcaaccgtggctccctcactttctggctggatgatggggcgattcaggcctggtatgagtcagcaacaccttcttcacgaggcagacctcagcgcccccccccccctagcttgtctacgtctgatgctttgaatcggacggacttgccgatcttgtatgcggtgatttttccctcgtttgcccactttttaatggtggccggggtgagagctacgcgggcggcgacctgctgcgctgtgatccaatattcggggtcgttcactggttcccctttctgatttctggcatagaagaacccccgtgaactgtgtggttccgggggttgctgatttttgcgagacttctcgcgcaattccctagcttaggtgaaaacaccatgaaacactagggaaacacccatgaaacacccattagggcagtagggcggcttcttcgtctagggcttgcatttgggcggtgatctggtctttagcgtgtgaaagtgtgtcgtaggtggcgtgctcaatgcactcgaacgtcacgtcatttaccgggtcacggtgggcaaagagaactagtgggttagacattgttttcctcgttgtcggtggtggtgagcttttctagccgctcggtaaacgcggcgatcatgaactcttggaggttttcaccgttctgcatgcctgcgcgcttcatgtcctcacgtagtgccaaaggaacgcgtgcggtgaccacgacgggcttagcctttgcctgcgcttctagtgcttcgatggtggcttgtgcctgcgcttgctgcgcctgtagtgcctgttgagcttcttgtagttgctgttctagctgtgccttggttgccatgctttaagactctagtagctttcctgcgatatgtcatgcgcatgcgtagcaaacattgtcctgcaactcattcattatgtgcagtgctcctgttactagtcgtacatactcatatttacctagtctgcatgcagtgcatgcacatgcagtcatgtcgtgctaatgtgtaaaacatgtacatgcagattgctgggggtgcagggggcggagccaccctgtccatgcggggtgtggggcttgccccgccggtacagacagtgagcaccggggcacctagtcgcggataccccccctaggtatcggacacgtaaccctcccatgtcgatgcaaatctttaacattgagtacgggtaagctggcacgcatagccaagctaggcggccaccaaacaccactaaaaattaatagttcctagacaagacaaacccccgtgcgagctaccaactcatatgcacgggggccacataacccgaaggggtttcaattgacaaccatagcactagctaagacaacgggcacaacacccgcacaaactcgcactgcgcaaccccgcacaacatcgggtctaggtaacactgaaatagaagtgaacacctctaaggaaccgcaggtcaatgagggttctaaggtcactcgcgctagggcgtggcgtaggcaaaacgtcatgtacaagatcaccaatagtaaggctctggcggggtgccataggtggcgcagggacgaagctgttgcggtgtcctggtcgtctaacggtgcttcgcagtttgagggtctgcaaaactctcactctcgctgggggtcacctctggctgaattggaagtcatgggcgaacgccgcattgagctggctattgctactaagaatcacttggcggcgggtggcgcgctcatgatgtttgtgggcactgttcgacacaaccgctcacagtcatttgcgcaggttgaagcgggtattaagactgcgtactcttcgatggtgaaaacatctcagtggaagaaagaacgtgcacggtacggggtggagcacacctatagtgactatgaggtcacagactcttgggcgaacggttggcacttgcaccgcaacatgctgttgttcttggatcgtccactgtctgacgatgaactcaaggcgtttgaggattccatgttttcccgctggtctgctggtgtggttaaggccggtatggacgcgccactgcgtgagcacggggtcaaacttgatcaggtgtctacctggggtggagacgctgcgaaaatggcaacctacctcgctaagggcatgtctcaggaactgactggctccgctactaaaaccgcgtctaaggggtcgtacacgccgtttcagatgttggatatgttggccgatcaaagcgacgccggcgaggatatggacgctgttttggtggctcggtggcgtgagtatgaggttggttctaaaaacctgcgttcgtcctggtcacgtggggctaagcgtgctttgggcattgattacatagacgctgatgtacgtcgtgaaatggaagaagaactgtacaagctcgccggtctggaagcaccggaacgggtcgaatcaacccgcgttgctgttgctttggtgaagcccgatgattggaaactgattcagtctgatttcgcggttaggcagtacgttctagattgcgtggataaggctaaggacgtggccgctgcgcaacgtgtcgctaatgaggtgctggcaagtctgggtgtggattccaccccgtgcatgatcgttatggatgatgtggacttggacgcggttctgcctactcatggggacgctactaagcgtgatctgaatgcggcggtgttcgcgggtaatgagcagactattcttcgcacccactaaaagcggcataaaccccgttcgatattttgtgcgatgaatttatggtcaatgtcgcgggggcaaactatgatgggtcttgttgttgacaatggctgatttcatcaggaatggaactgtcatgctgttatgtgcctggctcctaatcaaagctggggacaatgggttgccccgttgatctgatctagttcggattggcggggcttcactgtatctgggggtggcatcgtgaatagattgcacaccgtagtgggcagtgtgcacaccatagtggccatgagcaccaccacccccagggacgccgacggcgcgaagctctgcgcctggtgcggctcggagatcaagcaatccggcgtcggccggagccgggactactgccgccgctcctgccgccagcgggcgtacgaggcccggcgccagcgcgaggcgatcgtgtccgccgtggcgtcggcagtcgctcgccgagatacgtcacgtgacgaaatgcagcagccttccattccgtcacgtgacgaaactcgggccgcaggtcagagcacggttccgcccgctccggccctgccggacccccggcatcccgcaagaggcccggcagtaccggcataaccaagcctatgcctacagcatccagggtgacggtgccgaggatgacgatgagcgcattgttagatttcatacacggtgcctgactgcgttagcaatttaactgtgataaactaccgcattaaagcttatcgatgataagctgtcaaacatggcctgtcgcttgcggtattcggaatcttgcacgccctcgctcactgcccgctttccagtcgggaaacctgtcgtgccagctgcattaatgaatcggccaacgcgcggggagaggcggtttgcgtattgggcgccagggtggtttttcttttcaccagtgagacgggcaacagctgattgcccttcaccgcctggccctgagagagttgcagcaagcggtccacgctggtttgccccagcaggcgaaaatcctgtttgatggtggttaacggcgggatataacatgagctgtcttcggtatcgtcgtatcccactaccgagatatccgcaccaacgcgcagcccggactcggtaatggcgcgcattgcgcccagcgccatctgatcgttggcaaccagcatcgcagtgggaacgatgccctcattcagcatttgcatggtttgttgaaaaccggacatggcactccagtcgccttcccgttccgctatcggctgaatttgattgcgagtgagatatttatgccagccagccagacgcagacgcgccgagacagaacttaatgggcccgctaacagcgcgatttgctggtgacccaatgcgaccagatgctccacgcccagtcgcgtaccgtcttcatgggagaaaataatactgttgatgggtgtctggtcagagacatcaagaaataacgccggaacattagtgcaggcagcttccacagcaatggcatcctggtcatccagcggatagttaatgatcagcccactgacgcgttgcgcgagaagattgtgcaccgccgctttacaggcttcgacgccgcttcgttctaccatcgacaccaccacgctggcacccagttgatcggcgcgagatttaatcgccgcgacaatttgcgacggcgcgtgcagggccagactggaggtggcaacgccaatcagcaacgactgtttgcccgccagttgttgtgccacgcggttgggaatgtaattcagctccgccatcgccgcttccactttttcccgcgttttcgcagaaacgtggctggcctggttcaccacgcgggaaacggtctgataagagacaccggcatactctgcgacatcgtataacgttactggtttcacattcaccaccctgaattgactctcttccgggcgctatcatgccataccgcgaaaggttttgcaccattcgatggtgtcaacgtaaatgcatgccgcttcgccttcgcgcgcgaattgcaagctgatccgggcttatcgactgcacggtgcaccaatgcttctggcgtcaggcagccatcggaagctgtggtatggctgtgcaggtcgtaaatcactgcataattcgtgtcgctcaaggcgcactcccgttctggataatgttttttgcgccgacatcataacggttctggcaaatattctgaaatgagctgttgacaattaatcatcggctcgtataatgtgtggaattgtgagcggataacaatttcacacaggaaacagaattaaaagatatgaccatgattacgccaagcttgcatgcctgcaggtcgac

SEQ ID NO: 5 - DNA, 75 bp, Corynebacterium ammoniagenes
  source 1..75: mol_type = other DNA
atgaaacgcatgaaatcgctggctgcggcgctcaccgtcgctggggccatgctggccgcacctgtggcaacggca

SEQ ID NO: 6 - DNA, 9612 bp, synthetic construct
  source 1..9612: mol_type = other DNA
atgaaacgcatgaaatcgctggctgcggcgctcaccgtcgctggggccatgctggccgcacctgtggcaacggcaggcgctgacgacgttgttgactcctccaagtccttcgttatggagaacttctcctcctaccacggcaccaagccaggctacgttgactccatccagaagggcatccagaagccaaagtccggcacccagggcaactacgacgacgactggaaggagttctactccaccgacaacaagtacgacgctgctggctactccgttgacaacgagaacccactgtccggcaaggctggcggcgttgttaaggttacctacccaggcctgaccaaggttctggctctgaaggttgacaacgctgagaccatcaagaaggagctgggcctgtccctgaccgagccactgatggagcaggttggcaccgaggagttcatcaagcgcttcggcgacggcgcttcccgcgttgttctgtccctgccattcgctgagggctcctcctccgttgagtacatcaacaactgggagcaggctaaggctctgtccgttgagctggagatcaacttcgagacccgcggcaagcgcggccaggacgctatgtacgagtacatggctcaggcttgcgctggcaaccgcgttcgccgctccgttggctcctccctgtcctgcatcaacctggactgggacgttatccgcgacaagaccaagaccaagatcgagtccctgaaggagcacggcccaatcaagaacaagatgtccgagtccccaaacaagaccgtttccgaggagaaggctaagcagtacctggaggagttccaccagaccgctctggagcacccagagctgtccgagctgaagaccgttaccggcaccaacccagttttcgctggcgctaactacgctgcttgggctgttaacgttgctcaggttatcgactccgagaccgctgacaacctggagaagaccaccgctgctctgtccatcctgccaggcatcggctccgttatgggcatcgctgacggcgctgttcaccacaacaccgaggagatcgttgctcagtccatcgctctgtcctccctgatggttgctcaggctatcccactggttggcgagctggttgacatcggcttcgctgcttacaacttcgttgagtccatcatcaacctgttccaggttgttcacaactcctacaaccgcccagcttactccccaggccacaagacccagccattcctgcacgacgggtacgctgtcagctggaacaccgttgaggactccatcatccgcaccggcttccagggcgagtccggccacgacatcaagatcaccgctgagaacaccccactgccaatcgctggcgttctgctgccaaccatcccaggcaagctggacgttaacaagtccaagacccacatctccgttaacggccgcaagatccgcatgcgctgccgcgctatcgacggcgacgttaccttctgccgcccaaagtccccagtttacgttggcaacggcgttcacgctaacctgcacgttgctttccaccgctcctcctccgagaagatccactccaacgagatctcctccgactccatcggcgttctgggctaccagaagaccgttgaccacaccaaggttaactccaagctgtccctgttcttcgagatcaagtcctaaggatccccgggtaccgagctcgaatacactggccgtcgttttacagccaagcttggctgttttggcggatgagagaagattttcagcctgatacagattaaatcagaacgcagaagcggtctgataaaacagaatttgcctggcggcagtagcgcggtggtcccacctgaccccatgccgaactcagaagtgaaacgccgtagcgccgatggtagtgtggggtctccccatgcgagagtagggaactgccaggcatcaaataaaacgaaaggctcagtcgaaagactgggcctttcgttttatctgttgtttgtcggtgaacgctctcctgagtaggacaaatccgccgggagcggatttgaacgttgcgaagcaacggcccggagggtggcgggcaggacgcccgccataaactgccaggcatcaaattaagcagaaggccatcctgacggatggcctttttgcgtttctacaaactcttttgtttatttttctaaatacattcaaatatgtatccgctcatgagacaataaccctgataaatgcttcaataatattgaaaaaggaagagtatgagtattcaacatttccgtgtcgcccttattcccttttttgcggcattttgccttcctgtttttgctcacccagaaacgctggtgaaagtaaaagatgctgaagatcagttgggtgcacgagtgggttacatcgaactggatctcaacagcggtaagatccttgagagttttcgccccgaagaacgttttccaatgatgagcacttttaaagttctgctatgtggcgcggtattatcccgtgttgacgccgggcaagagcaactcggtcgccgcatacactattctcagaatgacttggttgagtaattcgtaatcatgtcataggctcttccgcttcctcgctcactgactcgctgcgctcggtcgttcggctgcggcgagcggtatcagctcactcaaaggcggtaatacggttatccacagaatcaggggataacgcaggaaagaacatgtgagcaaaaggccagcaaaaggccaggaaccgtaaaaaggccgcgttgctggcgtttttccataggctccgcccccctgacgagcatcacaaaaatcgacgctcaagtcagaggtggcgaaacccgacaggactataaagataccaggcgtttccccctggaagctccctcgtgcgctctcctgttccgaccctgccgcttaccggatacctgtccgcctttctcccttcgggaagcgtggcgctttctcatagctcacgctgtaggtatctcagttcggtgtaggtcgttcgctccaagctgggctgtgtgcacgaaccccccgttcagcccgaccgctgcgccttatccggtaactatcgtcttgagtccaacccggtaagacacgacttatcgccactggcagcagccactggtaacaggattagcagagcgaggtatgtaggcggtgctacagagttcttgaagtggtggcctaactacggctacactagaagaacagtatttggtatctgcgctctgctgaagccagttaccttcggaaaaagagttggtagctcttgatccggcaaacaaaccaccgctggtagcggtggtttttttgtttgcaagcagcagattacgcgcagaaaaaaaggatctcaagaagatcctttgatcttttctacggggtctgacgctcagtggaacgaaaactcacgttaagggattttggtcatgagattatcaaaaaggatcttcacctagatccttttggggggggggggaaagccacgttgtgtctcaaaatctctgatgttacattgcacaagataaaaatatatcatcatgaacaataaaactgtctgcttacataaacagtaatacaaggggtgttatgagccatattcaacgggaaacgtcttgctcgaggccgcgattaaattccaacatggatgctgatttatatgggtataaatgggctcgcgataatgtcgggcaatcaggtgcgacaatctatcgattgtatgggaagcccgatgcgccagagttgtttctgaaacatggcaaaggtagcgttgccaatgatgttacagatgagatggtcagactaaactggctgacggaatttatgcctcttccgaccatcaagcattttatccgtactcctgatgatgcatggttactcaccactgcgatccccgggaaaacagcattccaggtattagaagaatatcctgattcaggtgaaaatattgttgatgcgctggcagtgttcctgcgccggttgcattcgattcctgtttgtaattgtccttttaacagcgatcgcgtatttcgtctcgctcaggcgcaatcacgaatgaataacggtttggttgatgcgagtgattttgatgacgagcgtaatggctggcctgttgaacaagtctggaaagaaatgcataagcttttgccattctcaccggattcagtcgtcactcatggtgatttctcacttgataaccttatttttgacgaggggaaattaataggttgtattgatgttggacgagtcggaatcgcagaccgataccaggatcttgccatcctatggaactgcctcggtgagttttctccttcattacagaaacggctttttcaaaaatatggtattgataatcctgatatgaataaattgcagtttcatttgatgctcgatgagtttttctaatcagaattggttaattggttgtaacactggcagagcattacgctgacttgacgggacggcggctttgttgaataaatcgaacttttgctgagttgaaggatcagatcacgcatcttcccgacaacgcagaccgttccgtggcaaagcaaaagttcaaaatcaccaactggtccacctacaacaaagctctcatcaaccgtggctccctcactttctggctggatgatggggcgattcaggcctggtatgagtcagcaacaccttcttcacgaggcagacctcagcgcccccccccccctagcttgtctacgtctgatgctttgaatcggacggacttgccgatcttgtatgcggtgatttttccctcgtttgcccactttttaatggtggccggggtgagagctacgcgggcggcgacctgctgcgctgtgatccaatattcggggtcgttcactggttcccctttctgatttctggcatagaagaacccccgtgaactgtgtggttccgggggttgctgatttttgcgagacttctcgcgcaattccctagcttaggtgaaaacaccatgaaacactagggaaacacccatgaaacacccattagggcagtagggcggcttcttcgtctagggcttgcatttgggcggtgatctggtctttagcgtgtgaaagtgtgtcgtaggtggcgtgctcaatgcactcgaacgtcacgtcatttaccgggtcacggtgggcaaagagaactagtgggttagacattgttttcctcgttgtcggtggtggtgagcttttctagccgctcggtaaacgcggcgatcatgaactcttggaggttttcaccgttctgcatgcctgcgcgcttcatgtcctcacgtagtgccaaaggaacgcgtgcggtgaccacgacgggcttagcctttgcctgcgcttctagtgcttcgatggtggcttgtgcctgcgcttgctgcgcctgtagtgcctgttgagcttcttgtagttgctgttctagctgtgccttggttgccatgctttaagactctagtagctttcctgcgatatgtcatgcgcatgcgtagcaaacattgtcctgcaactcattcattatgtgcagtgctcctgttactagtcgtacatactcatatttacctagtctgcatgcagtgcatgcacatgcagtcatgtcgtgctaatgtgtaaaacatgtacatgcagattgctgggggtgcagggggcggagccaccctgtccatgcggggtgtggggcttgccccgccggtacagacagtgagcaccggggcacctagtcgcggataccccccctaggtatcggacacgtaaccctcccatgtcgatgcaaatctttaacattgagtacgggtaagctggcacgcatagccaagctaggcggccaccaaacaccactaaaaattaatagttcctagacaagacaaacccccgtgcgagctaccaactcatatgcacgggggccacataacccgaaggggtttcaattgacaaccatagcactagctaagacaacgggcacaacacccgcacaaactcgcactgcgcaaccccgcacaacatcgggtctaggtaacactgaaatagaagtgaacacctctaaggaaccgcaggtcaatgagggttctaaggtcactcgcgctagggcgtggcgtaggcaaaacgtcatgtacaagatcaccaatagtaaggctctggcggggtgccataggtggcgcagggacgaagctgttgcggtgtcctggtcgtctaacggtgcttcgcagtttgagggtctgcaaaactctcactctcgctgggggtcacctctggctgaattggaagtcatgggcgaacgccgcattgagctggctattgctactaagaatcacttggcggcgggtggcgcgctcatgatgtttgtgggcactgttcgacacaaccgctcacagtcatttgcgcaggttgaagcgggtattaagactgcgtactcttcgatggtgaaaacatctcagtggaagaaagaacgtgcacggtacggggtggagcacacctatagtgactatgaggtcacagactcttgggcgaacggttggcacttgcaccgcaacatgctgttgttcttggatcgtccactgtctgacgatgaactcaaggcgtttgaggattccatgttttcccgctggtctgctggtgtggttaaggccggtatggacgcgccactgcgtgagcacggggtcaaacttgatcaggtgtctacctggggtggagacgctgcgaaaatggcaacctacctcgctaagggcatgtctcaggaactgactggctccgctactaaaaccgcgtctaaggggtcgtacacgccgtttcagatgttggatatgttggccgatcaaagcgacgccggcgaggatatggacgctgttttggtggctcggtggcgtgagtatgaggttggttctaaaaacctgcgttcgtcctggtcacgtggggctaagcgtgctttgggcattgattacatagacgctgatgtacgtcgtgaaatggaagaagaactgtacaagctcgccggtctggaagcaccggaacgggtcgaatcaacccgcgttgctgttgctttggtgaagcccgatgattggaaactgattcagtctgatttcgcggttaggcagtacgttctagattgcgtggataaggctaaggacgtggccgctgcgcaacgtgtcgctaatgaggtgctggcaagtctgggtgtggattccaccccgtgcatgatcgttatggatgatgtggacttggacgcggttctgcctactcatggggacgctactaagcgtgatctgaatgcggcggtgttcgcgggtaatgagcagactattcttcgcacccactaaaagcggcataaaccccgttcgatattttgtgcgatgaatttatggtcaatgtcgcgggggcaaactatgatgggtcttgttgttgacaatggctgatttcatcaggaatggaactgtcatgctgttatgtgcctggctcctaatcaaagctggggacaatgggttgccccgttgatctgatctagttcggattggcggggcttcactgtatctgggggtggcatcgtgaatagattgcacaccgtagtgggcagtgtgcacaccatagtggccatgagcaccaccacccccagggacgccgacggcgcgaagctctgcgcctggtgcggctcggagatcaagcaatccggcgtcggccggagccgggactactgccgccgctcctgccgccagcgggcgtacgaggcccggcgccagcgcgaggcgatcgtgtccgccgtggcgtcggcagtcgctcgccgagatacgtcacgtgacgaaatgcagcagccttccattccgtcacgtgacgaaactcgggccgcaggtcagagcacggttccgcccgctccggccctgccggacccccggcatcccgcaagaggcccggcagtaccggcataaccaagcctatgcctacagcatccagggtgacggtgccgaggatgacgatgagcgcattgttagatttcatacacggtgcctgactgcgttagcaatttaactgtgataaactaccgcattaaagcttatcgatgataagctgtcaaacatggcctgtcgcttgcggtattcggaatcttgcacgccctcgctcactgcccgctttccagtcgggaaacctgtcgtgccagctgcattaatgaatcggccaacgcgcggggagaggcggtttgcgtattgggcgccagggtggtttttcttttcaccagtgagacgggcaacagctgattgcccttcaccgcctggccctgagagagttgcagcaagcggtccacgctggtttgccccagcaggcgaaaatcctgtttgatggtggttaacggcgggatataacatgagctgtcttcggtatcgtcgtatcccactaccgagatatccgcaccaacgcgcagcccggactcggtaatggcgcgcattgcgcccagcgccatctgatcgttggcaaccagcatcgcagtgggaacgatgccctcattcagcatttgcatggtttgttgaaaaccggacatggcactccagtcgccttcccgttccgctatcggctgaatttgattgcgagtgagatatttatgccagccagccagacgcagacgcgccgagacagaacttaatgggcccgctaacagcgcgatttgctggtgacccaatgcgaccagatgctccacgcccagtcgcgtaccgtcttcatgggagaaaataatactgttgatgggtgtctggtcagagacatcaagaaataacgccggaacattagtgcaggcagcttccacagcaatggcatcctggtcatccagcggatagttaatgatcagcccactgacgcgttgcgcgagaagattgtgcaccgccgctttacaggcttcgacgccgcttcgttctaccatcgacaccaccacgctggcacccagttgatcggcgcgagatttaatcgccgcgacaatttgcgacggcgcgtgcagggccagactggaggtggcaacgccaatcagcaacgactgtttgcccgccagttgttgtgccacgcggttgggaatgtaattcagctccgccatcgccgcttccactttttcccgcgttttcgcagaaacgtggctggcctggttcaccacgcgggaaacggtctgataagagacaccggcatactctgcgacatcgtataacgttactggtttcacattcaccaccctgaattgactctcttccgggcgctatcatgccataccgcgaaaggttttgcaccattcgatggtgtcaacgtaaatgcatgccgcttcgccttcgcgcgcgaattgcaagctgatccgggcttatcgactgcacggtgcaccaatgcttctggcgtcaggcagccatcggaagctgtggtatggctgtgcaggtcgtaaatcactgcataattcgtgtcgctcaaggcgcactcccgttctggataatgttttttgcgccgacatcataacggttctggcaaatattctgaaatgagctgttgacaattaatcatcggctcgtataatgtgtggaattgtgagcggataacaatttcacacaggaaacagaattaaaagatatgaccatgattacgccaagcttgcatgcctgcaggtcgac

SEQ ID NO: 7 - DNA, 1605 bp, synthetic construct
  source 1..1605: mol_type = other DNA
ggcgctgatgatgttgttgattcttctaagtctttcgtgatggaaaacttctcttcctaccacggcactaagcctggttacgttgattccattcagaagggtatccagaagccaaagtctggtacccagggcaactacgacgatgattggaaggagttctactccaccgacaacaagtacgacgctgctggctactctgtagataacgaaaacccactctctggcaaggctggcggcgtggtcaaggtgacctacccaggcctgaccaaggttctcgcactgaaggtggataacgctgaaactattaagaaggagctgggtctgtccctcactgaaccactgatggagcaggtcggcaccgaagagttcatcaagcgcttcggtgatggtgcttcccgtgtagtgctctcccttccattcgctgagggctcctcttccgttgaatacattaacaactgggaacaggctaaggctctgtccgtagaacttgagattaacttcgaaacccgtggcaagcgtggccaggatgctatgtacgagtacatggctcaggcttgtgcaggcaaccgtgtccgccgctccgtaggttcctccctgtcctgcatcaaccttgattgggatgtcatccgcgataagactaagaccaagatcgagtctctgaaggagcacggccctatcaagaacaagatgtccgaatccccaaacaagaccgtatctgaggaaaaggctaagcagtacctggaagagttccaccagaccgcactggagcaccctgaactgtccgaacttaagaccgttactggcaccaaccctgtattcgctggcgctaactacgctgcttgggcagtaaacgttgctcaggttatcgattccgaaaccgctgataacctggaaaagaccactgctgctctttccatccttcctggtatcggttccgtaatgggcattgcagacggtgctgttcaccacaacaccgaagagatcgtggcacagtccatcgctctgtcctctctgatggttgctcaggctattccactggtaggcgagctggttgatattggtttcgctgcatacaacttcgtagagtccattatcaacctgttccaggtagttcacaactcctacaaccgtccagcttactctccaggccacaagacccagccattccttcacgacggctacgctgtctcctggaacactgttgaagattccatcatccgcactggtttccagggcgagtccggccacgacatcaagattactgctgaaaacaccccacttccaatcgctggtgtcctgctgccaactattcctggcaagctggacgttaacaagtccaagactcacatttccgtaaacggtcgcaagatccgcatgcgttgccgcgctatcgacggcgacgtaacattctgtcgccctaagtctcctgtttacgttggtaacggtgtgcacgctaaccttcacgtggcattccaccgctcctcctccgagaagattcactctaacgaaatttcctccgattccatcggcgttcttggctaccagaagaccgtagatcacaccaaggttaactctaagctgtccctgttcttcgaaatcaagtcc

SEQ ID NO: 8 - DNA, 1605 bp, synthetic construct
  source 1..1605: mol_type = other DNA
ggcgcggatgatgtggtggatagcagcaaaagctttgtgatggaaaactttagcagctatcatggcaccaaaccgggctatgtggatagcattcagaaaggcattcagaaaccgaaaagcggcacccagggcaactatgatgatgattggaaagaattttatagcaccgataacaaatatgatgcggcgggctatagcgtggataacgaaaacccgctgagcggcaaagcgggcggcgtggtgaaagtgacctatccgggcctgaccaaagtgctggcgctgaaagtggataacgcggaaaccattaaaaaagaactgggcctgagcctgaccgaaccgctgatggaacaggtgggcaccgaagaatttattaaacgctttggcgatggcgcgagccgcgtggtgctgagcctgccgtttgcggaaggcagcagcagcgtggaatatattaacaactgggaacaggcgaaagcgctgagcgtggaactggaaattaactttgaaacccgcggcaaacgcggccaggatgcgatgtatgaatatatggcgcaggcgtgcgcgggcaaccgcgtgcgccgcagcgtgggcagcagcctgagctgcattaacctggattgggatgtgattcgcgataaaaccaaaaccaaaattgaaagcctgaaagaacatggcccgattaaaaacaaaatgagcgaaagcccgaacaaaaccgtgagcgaagaaaaagcgaaacagtatctggaagaatttcatcagaccgcgctggaacatccggaactgagcgaactgaaaaccgtgaccggcaccaacccggtgtttgcgggcgcgaactatgcggcgtgggcggtgaacgtggcgcaggtgattgatagcgaaaccgcggataacctggaaaaaaccaccgcggcgctgagcattctgccgggcattggcagcgtgatgggcattgcggatggcgcggtgcatcataacaccgaagaaattgtggcgcagagcattgcgctgagcagcctgatggtggcgcaggcgattccgctggtgggcgaactggtggatattggctttgcggcgtataactttgtggaaagcattattaacctgtttcaggtggtgcataacagctataaccgcccggcgtatagcccgggccataaaacccagccgtttctgcatgatggctatgcggtgagctggaacaccgtggaagatagcattattcgcaccggctttcagggcgaaagcggccatgatattaaaattaccgcggaaaacaccccgctgccgattgcgggcgtgctgctgccgaccattccgggcaaactggatgtgaacaaaagcaaaacccatattagcgtgaacggccgcaaaattcgcatgcgctgccgcgcgattgatggcgatgtgaccttttgccgcccgaaaagcccggtgtatgtgggcaacggcgtgcatgcgaacctgcatgtggcgtttcatcgcagcagcagcgaaaaaattcatagcaacgaaattagcagcgatagcattggcgtgctgggctatcagaaaaccgtggatcataccaaagtgaacagcaaactgagcctgttttttgaaattaaaagc